European Patent Application EP 4 342 989 A1, published March 27, 2024. Title: Anti-norovirus antibody. Applicant: DENKA COMPANY LIMITED. The sequence listing filed with the application follows.

SEQUENCE LISTING (4 sequences)

SEQ ID NO: 1 - protein, 23 aa, Artificial Sequence
  partial sequence of shell domain of capsid of norovirus
MMMASKDAPPSMDGASGAGQLVP

SEQ ID NO: 2 - protein, 21 aa, Artificial Sequence
  partial sequence of shell domain of capsid of norovirus
MKMASNDAAPSNDGAAGLVPE

SEQ ID NO: 3 - protein, 17 aa, Artificial Sequence
  partial sequence of shell domain of capsid of norovirus
MMMASKDAPPSMDGASG

SEQ ID NO: 4 - protein, 17 aa, Artificial Sequence
  partial sequence of shell domain of capsid of norovirus
MKMASNDAAPSNDGAAG